European Patent Application EP 4 737 557 A1, published May 6, 2026. Title: 改造的大肠杆菌及其在发酵生产L-氨基酸中的应用. Applicant: 宁夏伊品生物科技股份有限公司. Application CN. The sequence listing filed with the application follows.

SEQUENCE LISTING (54 sequences)

SEQ ID NO: 1 - DNA, 23 bp, synthetic construct
  source 1..23: mol_type = other DNA
gcgaatttcttgaagttcagcgg

SEQ ID NO: 2 - DNA, 1339 bp, synthetic construct
  source 1..1339: mol_type = other DNA
cgttggtgtccagacaggtatgaatgccttcttttttgcaggcgcggaaccagtcacgaacaaactcagcttgcaggattgcttcaccgccggatgcggtaacgccgccgccggaagcgttcataaagtggcgataggtcaccacttccttcatcaaatcttcaacggtaacttctttaccgccatgcgtgtcccaggtgtcgcggttatgacaatacaggcagcgcatcaggcagccctggaaaaaggtgataaagcgaatacctgggccgtctacggttccacaggattcaaaggagtgaatgcgaccaataactgacattgcggtgtttctccagatgtggcccatctgaggccgtgttggtgcgcagctcgaaggctacgtcgagtctgttttggcagtcaccttaaagtatagatagctgacaaaaaaggctctcgcgctaaaaaaggccccactttcgtggagcctttattgtacgctttttactgtacgatttcagtcaaatctaattacatagattgagtgaaggtacgagtaataacgtcctgctgctgttctttagtcagcgagttgaaacgtactgcgtagccagatacacggatggtcagctgcggatatttttccgggttttccatcgcgtcgagcagcatttcacggttcatttacggcaacgcaggatgtccggagtgtaaacgtcgaacacgccctggttgtgagttttacggtattcagtgaagatttttttgatcatcggatccagttcgcggttgtacgctttgcaggaaccttcgatcattttgataccaccgaacgggataagagcacgtttcagcggagcttcagtctgcagaccaacgattttctcaagctgcttgttgatgtagccagcgtcgtgagaggtgatggtggaagcaacagcggtgtcaaagtcaactggcgcgtgagtgcggttttccagtttaacgccttccattactttgtcccacagggtggtggtcgcttcagtagcgccagccaggaaggactcgtcaccctcgtacggagtgtagtttttctgaatgaagtcacggacgtttacttcattctgccagtcacctttggtaaaaccttcccaggctgtggctaacttttcattaagctcggacatgtaacacctaccttcttaagtggattttttatttactgcgtacttcgacaaccattaatggtggtcgttttcacgcaggtaaatgacccagtatgtcaacccaaccaacaaaccaccaccgataatgttgccgatcgtaaccggaatcaggttatcagtgatgaaattcatcacggtcaggtgagaaa

SEQ ID NO: 3 - DNA, 943 bp, synthetic construct
  source 1..943: mol_type = other DNA
gcagtggcggttttcatggcttgttatgactgtttttttggggtacagtctatgcctcgggcatccaagcagcaagcgcgttacgccgtgggtcgatgtttgatgttatggagcagcaacgatgttacgcagcagggcagtcgccctaaaacaaagttaaacatcatgagggaagcggtgatcgccgaagtatcgactcaactatcagaggtagttggcgtcatcgagcgccatctcgaaccgacgttgctggccgtacatttgtacggctccgcagtggatggcggcctgaagccacacagtgatattgatttgctggttacggtgaccgtaaggcttgatgaaacaacgcggcgagctttgatcaacgaccttttggaaacttcggcttcccctggagagagcgagattctccgcgctgtagaagtcaccattgttgtgcacgacgacatcattccgtggcgttatccagctaagcgcgaactgcaatttggagaatggcagcgcaatgacattcttgcaggtatcttcgagccagccacgatcgacattgatctggctatcttgctgacaaaagcaagagaacatagcgttgccttggtaggtccagcggcggaggaactctttgatccggttcctgaacaggatctatttgaggcgctaaatgaaaccttaacgctatggaactcgccgcccgactgggctggcgatgagcgaaatgtagtgcttacgttgtcccgcatttggtacagcgcagtaaccggcaaaatcgcgccgaaggatgtcgctgccgactgggcaatggagcgcctgccggcccagtatcagcccgtcatacttgaagctagacaggcttatcttggacaagaagaagatcgcttggcctcgcgcgcagatcagttggaagaatttgtccactacgtgaaaggcgagatcaccaagg

SEQ ID NO: 4 - DNA, 23 bp, synthetic construct
  source 1..23: mol_type = other DNA
aagaaccacaacccagagtcagg

SEQ ID NO: 5 - DNA, 1365 bp, synthetic construct
  source 1..1365: mol_type = other DNA
gtgccagtcatccttcaggtaacgttccgcgcccctgtctgtgcggtctggcggaagagccattccactggggcggcccccacgcgctgacgcgcctgggtgacagcgctgcgggccagcaggttcatccccgcttcgccatccgcgctcaggttcagacggcgaacaacatcggtaattggctcattgcaccaccatccagataaccatgtcccccggtaaacgacggcggcgaacggtcgcatgagcagaaagcgtcaggcagtgttgtatccactcggtgggaaggtgttctgcaaatagttgtgcagagggcggaggcataagcggatggtcactgaaatcgagcagatcattgagaagtggcataagaaaacggctccctgttgtggaagccgttatagtgcctcagtttaaggatcggtcaactaatccttaactgatcggcattgcccagaaggggccgtttatgttgccagacagcgctactgattaagcggattttttcgcttttttctcagctttagccggagcagcttctttcttcgctgcagtttcaccttctacataatcacgaccgtagtaggtatccagcagaatctgtttcagctcggagatcagcgggtaacgcgggttagcgccggtgcactggtcatcgaatgcatcttcagacagtttatccacgttcgccaggaagtctgcttcctgaacgccagcttcacggatagatttcggaatacccaagtcgggttagtggtcggaacgataccgcaaataataccgattggttcagcgatagtgatggtaccaaaagtgtcgtcttcagacagaacaccacaggttttttcatctttataggcgttgtagatatattcagaagcaaagtggtttttgatcactttatcttcgacgatacccatgccggattcggcaacggccattttcgcgagtgggattcgagcatctgcagcagccagagcggcggcgcggaagattttgtctacttgctcttgagtgaaactggcatattcacgctgggctttttttacacgctctacgagtgcgttaagttcagcgacattagtaacagccataatgctctcctgataatgttaaacttttttagtaaatcatctgctcgaatacgagagtatagtcagtgcggtgatgatttgcttaacctatgaaaatcaaaagcttactcgcgctcacactcactgtgatttactaaaagagtttaaacattagagttattatctctaatgcgtcacttccaggtggcgtaagcaagattactcacttctgggtactgattacgtgatccaaatcaaatttttgcaaagctgacacctttcagcatcgctt

SEQ ID NO: 6 - DNA, 1169 bp, synthetic construct
  source 1..1169: mol_type = other DNA
ttaacgtctgcttaatacactgtggccgttttgcaaaaactggcttcttgagcggcgcatgcgttcaatccgttcctctgctaagcggtcagccgctaaatatgcaggaatgccgtcacgctgagaaatctcaagtacacgctcgatattgccgtaaatgccttcaacttttttcaatgcacgttctgcattatagccgtaaagctcatctgccacgttgatgacaccgcccgcgttaatcacgtaatccggtgcataaacgatgcccatttcgtgaatttgatcaccatggcgtgtctcttttaattggttgttagccgcacctgcgatcactttcgccttcagctgtttaatggtgtcgtcgttaatagtcgcaccaagggcacacggcgcataaatatcgcagtcttgtgaataaatgtcatcaggatctaccgcacgggcgccaaaatcttcaactgcacgctgtacagattgtttgttgatatccgtaacgattaagtttgctccttcttcatgcaggtggcggcaaaggttataggctacgttcccaacaccctgtacagcaatggtttttccttcaagagagtcggttccgaaagcagctttagctgctgccttcattcctctgtacaccccgtacgctgtgactggggacggatttccagaagagccgaaagcaggagaaatccctgtgacatagtctgtctcatcatgaatgatatccatatcctcgaccgttgtgcccacatcttcagccgtgatgtatctgccattcagtccttgaatatagcggccaaacgcgcggaacatttcctcatttttgtctttgcgcggatcgccgataatgactgtttttccgccgccaaggtttaagcctgccgccgcgttcttataggtcatgcctcttgccaatctgagcgcatcttcaattgccgcttcttcattttcatatgtccacattctcgttccgccaagcgccggaccaagcgttgtatcatgaatggcgataatcgcttttaatccagattgttcatcctggcagaataccaattgttcgtaatcgtatttctccatatatttaaaaagttccatggtctgtttcctgtgtgaaattgttatccgctcacaattccacacattatacgagccggatgattaattgtcaa

SEQ ID NO: 7 - DNA, 23 bp, synthetic construct
  source 1..23: mol_type = other DNA
gaaagcagcgataatcacgtcgg

SEQ ID NO: 8 - DNA, 2413 bp, synthetic construct
  source 1..2413: mol_type = other DNA
caggcagttcattgagttagcggtaaacatcccggagcaggaaccgcaggtcggacacgcggaacgttcaacctgatcgctctgggagtcagatactttcgggtctgcgccctggatcatcgcatcaaccagatcgagcttgatgatctgatcggaaagtttggttttcccggcctccatcgggccgccggaaacaaagatcaccggaatattcaggcgcagggaagccatcagcatccccggggtgattttgtcgcagttagagatgcagaccatggcgtcggcgcagtgggcgttgaccatatactcaacggaatcagcgatcagttcgcgagatggcagtgaataaagcatccccccgtggcccatggcaatcccatcatccaccgcaatggtgttgaactctttggcaacgccgccagccgcttcaatttgttcggcgaccagtttaccgagatcgcgcagatggacgtgacccggtacaaattgggtgaacgagttcacaaccgcgataatcggcttaccgaaatcggcgtcggtcattccggtggcgcgccacagcgcacgagcacccgccatattacgaccatgagtggtggtggcggaacggtacttaggcatactttatttactcccagtgtctgtctcgtaaatgggacggtgcgtgccgtcccattttttgtatttaacgtctgcttaatacactgtggccgttttgcaaaaactggcttcttgagcggcgcatgcgttcaatccgttcctctgctaagcggtcagccgctaaatatgcaggaatgccgtcacgctgagaaatctcaagtacacgctcgatattgccgtaaatgccttcaacttttttcaatgcacgttctgcattatagccgtaaagctcatctgccacgttgatgacaccgcccgcgttaatcacgtaatccggtgcataaacgatgcccatttcgtgaatttgatcaccatggcgtgtctcttttaattggttgttagccgcacctgcgatcactttcgccttcagctgtttaatggtgtcgtcgttaatagtcgcaccaagggcacacggcgcataaatatcgcagtcttgtgaataaatgtcatcaggatctaccgcacgggcgccaaaatcttcaactgcacgctgtacagattgtttgttgatatccgtaacgattaagtttgctccttcttcatgcaggtggcggcaaaggttataggctacgttcccaacaccctgtacagcaatggtttttccttcaagagagtcggttccgaaagcagctttagctgctgccttcattcctctgtacaccccgtacgctgtgactggggacggatttccagaagagccgaaagcaggagaaatccctgtgacatagtctgtctcatcatgaatgatatccatatcctcgaccgttgtgcccacatcttcagccgtgatgtatctgccattcagtccttgaatatagcggccaaacgcgcggaacatttcctcatttttgtctttgcgcggatcgccgataatgactgtttttccgccgccaaggtttaagcctgccgccgcgttcttataggtcatgcctcttgccaatctgagcgcatcttcaattgccgcttcttcattttcatatgtccacattctcgttccgccaagcgccggaccaagcgttgtatcatgaatggcgataatcgcttttaatccagattgttcatcctggcagaataccaattgttcgtaatcgtatttctccatatatttaaaaagttccatggtctgtttcctgtgtgaaattgttatccgctcacaattccacacattatacgagccggatgattaattgtcaattttatattccttttgcgctcaggcgcggatttgttgtgatgtggttgtgctctggcagatggcaacgtgtgcgacgtccaccagtttatttaactgactaaacagtaagtcgaccgaccgtgggctggcaacggtcaattcgatatttatattttgtgcatcgctggcggcggccatattcattgagcagacgtggaaaccacgatgacgcaccacgcgtaaaacacgttctaaggtttctggattgaagcgagccgatacattgacctgatgttgcatcatgataatttctccaacatttctgaattactggcgccaggcggcaccagcggccagacgttctcaagttcgtcgattgagacatgaagcaggtatggcccatcactgttcagcatggtgtcgagtgccgcttcaacctggtctttccgggtgatgtgttggccatggatgccgaaggcgctggctaacatgaggaaatcggggttatcagtaagggtggtttcgctgtatcgttcctgaaaaaacagttgctgccattgtcgaaccatccctaaccgt

SEQ ID NO: 9 - DNA, 23 bp, synthetic construct
  source 1..23: mol_type = other DNA
cgcccctcttatatcgcgctggg

SEQ ID NO: 10 - DNA, 1296 bp, synthetic construct
  source 1..1296: mol_type = other DNA
ttctattcaggacgccaacgatgaagcgcagtttgccgagctgcatacgctgggcgaactgaccaaaattgcctgggaatatgacgtgcaggtgatgattgaaggcccaggccacgtgccgatgcagatgatccgccgcaatatgaccgaggagttagagcactgccacgaagcgccgttttacactctggggccgctaactaccgatattgcgccgggctatgaccacttcacgtcggggattggtgcggcgatgattggctggtttggctgcgcgatgctctgttacgtaacgccaaaagagcatctgggtctgcccaataaagaagatgttaagcaggggcttatcacctataagattgctgcccacgccgctgacctggcgaaagggcatccgggcgcgcaaattcgcgataacgccatgtcgaaagcccgcttcgaatttcgctgggaagaccagtttaatctggccctcgacccgtttaccgcccgcgcttatcacgatgaaaccctgccgcaagagtcaggtaaagtcgcccatttttgctccatgtgtgggccgaaattctgctcgatgaaaatcagccaggaagtgcgtgattacgccgccacgcaaactattgaaatgggaatggcggatatgtcggagaacttccgtgccagaggcggagaaatctacctgcgtaaggaggaagcgtgccgtgactttatgcgttatagccgccaaatcctgctcgacgatatcgctctggacgggcagcaaaaactgctcgacagccaggtgctgattatcggtctgggcgggctgggtacacctgctgcgctgtacctggcgggcgctggcgtcgggacgctggtactggcagatgacgacgatgtgcatttaagcaatctgcaacgacaaatcctctttaccactgaagatatcgatcgcccgaaatcgcaggtcagccaacagcgactgacacagttgaatcccgacattcaactgacagcattacaacaacggttaacgggtgaggcgttaaaagatgcggttgcacgggccgatgtggtgctcgactgtaccgacaatatggcgactcgccaggagattaatgccgcctgcgtggcactcaacacgccgcttatcaccgccagcgcggtcggatttggcggtcagttgatggtactgacgccgccctgggagcaggggtgttaccgctgcctgtggccagataaccaggagccagaacgcaactgccgcacggcgggcgtggttggcccggtggtcggggttatgggcactttgcaggc

SEQ ID NO: 11 - DNA, 23 bp, synthetic construct
  source 1..23: mol_type = other DNA
gcctttcagttccgcaacaaagg

SEQ ID NO: 12 - DNA, 1253 bp, synthetic construct
  source 1..1253: mol_type = other DNA
aacttcctccaaaccgatgcttccattaaccacggtaactctggcggcgcgctggtgaactcgctgggcgaactgatgggcattaatacgctgtcgtttgataagagtaacgatggcgaaacgccggaaggtatcggctttgcgattcctttccagttagcaaccaaaattatggataagctgatccgcgatggtcgcgtgatccgcggctacattggtatcggcggacgtgagatcgcaccactgcacgcgcagggcggtggtatagatcaactgcaagggatcgtggttaatgaagtgtcacctgacggcccggcggcgaatgcgggtattcaggtcaacgatctgattatttcggtggataacaaaccggccatctctgctctggagacgatggatcaggtggcggaaattcgccctggttcggtgatccctgtagtagtgatgcgtgatgataagcagttaacgctgcaggtcaccattcaggaatatccggcaaccaattaagtcgtgcgctcaaaacaaaaaaccggagtctgtgctccggttttttattatccgctaatcaacctaaactccttattatattgataaactaagatatgttgctccgctgccgcgaccttaatccacaaaattgccgtttacaatgaccacatctcaagaatgtgtagtcacgcaagtttagcgtttatgcatttaattgccgtaatcaggaacctaacttacgtaattaacagtcgcttatgcattagcgcaacattccaacaggtggtgacaatataccctaccgttcagccaaaacaacatcaatttgataacaattaatttacttttaagcagaatttgcatgccgtgacgcaggcatgtttctcaataacgaaatttgataaaatcccgctctttcataacattatttcagccttcttcagggctgactgtttgcataaaaattcatctgtatgcacaataatgttgtatcaaccaccatatcgggtgacttatgcgaagctcggctaagcaagaagaactagttaaagcatttaaagcattacttaaagaagagaaatttagctcccagggcgaaatcgtcgccgcgttgcaggagcaaggctttgacaatattaatcagtctaaagtctcgcggatgttgaccaagtttggtgctgtacgtacacgcaatgccaaaatggaaatggtttactgcctgccagctgaactgggtgtaccaaccacctccagtccattgaaga

SEQ ID NO: 13 - protein, 760 aa, synthetic construct
MSELNEKLATAWEGFTKGDWQNEVNVRDFIQKNYTPYEGDESFLAGATEATTTLWDKVMEGVKLENRTHAPVDFDTAVASTITSHDAGYINKQLEKIVGLQTEAPLKRALIPFGGIKMIEGSCKAYNRELDPMIKKIFTEYRKTHNQGVFDVYTPDILRCRKSGVLTGLPDAYGRGRIIGDYRRVALYGIDYLMKDKLAQFTSLQADLENGVNLEQTIRLREEIAEQHRALGQMKEMAAKYGYDISGPATNAQEAIQWTYFGYLAAVKSQNGAAMSFGRTSTFLDVYIERDLKAGKITEQEAQEMVDHLVMKLRMVRFLRTPEYDELFSGDPIWATESIGGMGLDGRTLVTKNSFRFLNTLYTMGPSPEPNMTILWSEKLPLNFKKFAAKVSIDTSSLQYENDDLMRPDFNNDDYAIACCVSPMIVGKQMQFFGARANLAKTMLYAINGGVDEKLKMQVGPKSEPIKGDVLNYDEVMERMDHFMDWLAKQYITALNIIHYMHDKYSYEASLMALHDRDVIRTMACGIAGLSVAADSLSAIKYAKVKPIRDEDGLAIDFEIEGEYPQFGNNDPRVDDLAVDLVERFMKKIQKLHTYRDAIPTQSVLTITSNVVYGKKTGNTPDGRRAGAPFGPGANPMHGRDQKGAVASLTSVAKLPFAYAKDGISYTFSIVPNALGKDDEVRKTNLAGLMDGYFHHEASIEGGQHLNVNVMNREMLLDAMENPEKYPQLTIRVSGYAVRFNSLTKEQQQDVITRTFTQSM

SEQ ID NO: 14 - protein, 891 aa, synthetic construct
MAVTNVAELNALVERVKKAQREYASFTQEQVDKIFRAAALAAADARIPLAKMAVAESGMGIVEDKVIKNHFASEYIYNAYKDEKTCGVLSEDDTFGTITIAEPIGIICGIVPTTNPTSTAIFKSLISLKTRNAIIFSPHPRAKDATNKAADIVLQAAIAAGAPKDLIGWIDQPSVELSNALMHHPDINLILATGGPGMVKAAYSSGKPAIGVGAGNTPVVIDETADIKRAVASVLMSKTFDNGVICASEQSVVVVDSVYDAVRERFATHGGYLLQGKELKAVQDVILKNGALNAAIVGQPAYKIAELAGFSVPENTKILIGEVTVVDESEPFAHEKLSPTLAMYRAKDFEDAVEKAEKLVAMGGIGHTSCLYTDQDNQPARVSYFGQKMKTARILINTPASQGGIGDLYNFKLAPSLTLGCGSWGGNSISENVGPKHLINKKTVAKRAENMLWHKLPKSIYFRRGSLPIALDEVITDGHKRALIVTDRFLFNNGYADQITSVLKAAGVETEVFFEVEADPTLSIVRKGAELANSFKPDVIIALGGGSPMDAAKIMWVMYEHPETHFEELALRFMDIRKRIYKFPKMGVKAKMIAVTTTSGTGSEVTPFAVVTDDATGQKYPLADYALTPDMAIVDANLVMDMPKSLCAFGGLDAVTHAMEAYVSVLASEFSDGQALQALKLLKEYLPASYHEGSKNPVARERVHSAATIAGIAFANAFLGVCHSMAHKLGSQFHIPHGLANALLICNVIRYNANDNPTKQTAFSQYDRPQARRRYAEIADHLGLSAPGDRTAAKIEKLLAWLETLKAELGIPKSIREAGVQEADFLANVDKLSEDAFDDQCTGANPRYPLISELKQILLDTYYGRDYVEGETAAKKEAAPAKAEKKAKKSA

SEQ ID NO: 15 - protein, 309 aa, synthetic construct
MTTKKADYIWFNGEMVRWEDAKVHVMSHALHYGTSVFEGIRCYDSHKGPVVFRHREHMQRLHDSAKIYRFPVSQSIDELMEACRDVIRKNNLTSAYIRPLIFVGDVGMGVNPPAGYSTDVIIAAFPWGAYLGAEALEQGIDAMVSSWNRAAPNTIPTAAKAGGNYLSSLLVGSEARRHGYQEGIALDVNGYISEGAGENLFEVKDGVLFTPPFTSSALPGITRDAIIKLAKELGIEVREQVLSRESLYLADEVFMSGTAAEITPVRSVDGIQVGEGRCGPVTKRIQQAFFGLFTGETEDKWGWLDQVNQ

SEQ ID NO: 16 - protein, 356 aa, synthetic construct
MNKLIEREKTVYYKEKPDPSSLGFGQYFTDYMFVMDYEEGIGWHHPRIAPYAPLTLDPSSSVFHYGQAVFEGLKAYRTDDGRVLLFRPDQNIKRLNRSCERMSMPPLDEELVLEALTQLVELEKDWVPKEKGTSLYIRPFVIATEPSLGVKASRSYTFMIVLSPVGSYYGDDQLKPVRIYVEDEYVRAVNGGVGFAKTAGNYAASLQAQRKANELGYDQVLWLDAIEKKYVEEVGSMNIFFVINGEAVTPALSGSILSGVTRASAIELIRSWGIPVREERISIDEVYAASARGELTEVFGTGTAAVVTPVGELNIHGKTVIVGDGQIGDLSKKLYETITDIQLGKVKGPFNWTVEV

SEQ ID NO: 17 - protein, 211 aa, synthetic construct
MYQPDFPPVPFRSGLYPVVDSVQWIERLLDAGVRTLQLRIKDRRDEEVEADVVAAIALGRRYNARLFINDYWRLAIKHQAYGVHLGQEDLQATDLNAIRAAGLRLGVSTHDDMEIDVALAARPSYIALGHVFPTQTKQMPSAPQGLEQLARHVERLADYPTVAIGGISLARAPAVIATGVGSIAVVSAITQAADWRLATAQLLEIAGVGDE

SEQ ID NO: 18 - protein, 312 aa, synthetic construct
MKVAVLGAAGGIGQALALLLKTQLPSGSELSLYDIAPVTPGVAVDLSHIPTAVKIKGFSGEDATPALEGADVVLISAGVARKPGMDRSDLFNVNAGIVKNLVQQVAKTCPKACIGIITNPVNTTVAIAAEVLKKAGVYDKNKLFGVTTLDIIRSNTFVAELKGKQPGEVEVPVIGGHSGVTILPLLSQVPGVSFTEQEVADLTKRIQNAGTEVVEAKAGGGSATLSMGQAAARFGLSLVRALQGEQGVVECAYVEGDGQYARFFSQPLLLGKNGVEERKSIGTLSAFEQNALEGMLDTLKKDIALGEEFVNK

SEQ ID NO: 19 - DNA, 91 bp, synthetic construct
  source 1..91: mol_type = other DNA
tgacagctagctcagtcctaggtataatactagtgcgaatttcttgaagttcagcgggttttagagctagaaatagcaagttaaaataagg

SEQ ID NO: 20 - DNA, 91 bp, synthetic construct
  source 1..91: mol_type = other DNA
ccttattttaacttgctatttctagctctaaaacccgctgaacttcaagaaattcgcactagtattatacctaggactgagctagctgtca

SEQ ID NO: 21 - DNA, 24 bp, synthetic construct
  source 1..24: mol_type = other DNA
gtctcatgagcggatacatatttg

SEQ ID NO: 22 - DNA, 18 bp, synthetic construct
  source 1..18: mol_type = other DNA
atgagaaagcgccacgct

SEQ ID NO: 23 - DNA, 22 bp, synthetic construct
  source 1..22: mol_type = other DNA
cgttggtgtccagacaggtatg

SEQ ID NO: 24 - DNA, 42 bp, synthetic construct
  source 1..42: mol_type = other DNA
gacatcctgcgttgccgtaaatgaaccgtgaaatgctgctcg

SEQ ID NO: 25 - DNA, 42 bp, synthetic construct
  source 1..42: mol_type = other DNA
cgagcagcatttcacggttcatttacggcaacgcaggatgtc

SEQ ID NO: 26 - DNA, 20 bp, synthetic construct
  source 1..20: mol_type = other DNA
tttctcacctgaccgtgatg

SEQ ID NO: 27 - DNA, 18 bp, synthetic construct
  source 1..18: mol_type = other DNA
gcagtggcggttttcatg

SEQ ID NO: 28 - DNA, 20 bp, synthetic construct
  source 1..20: mol_type = other DNA
ccttggtgatctcgcctttc

SEQ ID NO: 29 - DNA, 91 bp, synthetic construct
  source 1..91: mol_type = other DNA
tgacagctagctcagtcctaggtataatactagtaagaaccacaacccagagtcagggttttagagctagaaatagcaagttaaaataagg

SEQ ID NO: 30 - DNA, 91 bp, synthetic construct
  source 1..91: mol_type = other DNA
ccttattttaacttgctatttctagctctaaaaccctgactctgggttgtggttcttactagtattatacctaggactgagctagctgtca

SEQ ID NO: 31 - DNA, 20 bp, synthetic construct
  source 1..20: mol_type = other DNA
gtgccagtcatccttcaggt

SEQ ID NO: 32 - DNA, 43 bp, synthetic construct
  source 1..43: mol_type = other DNA
cgttccgaccactaacccgacttgggtattccgaaatctatcc

SEQ ID NO: 33 - DNA, 43 bp, synthetic construct
  source 1..43: mol_type = other DNA
ggatagatttcggaatacccaagtcgggttagtggtcggaacg

SEQ ID NO: 34 - DNA, 20 bp, synthetic construct
  source 1..20: mol_type = other DNA
aagcgatgctgaaaggtgtc

SEQ ID NO: 35 - DNA, 91 bp, synthetic construct
  source 1..91: mol_type = other DNA
tgacagctagctcagtcctaggtataatactagtgaaagcagcgataatcacgtcgggttttagagctagaaatagcaagttaaaataagg

SEQ ID NO: 36 - DNA, 91 bp, synthetic construct
  source 1..91: mol_type = other DNA
ccttattttaacttgctatttctagctctaaaacccgacgtgattatcgctgctttcactagtattatacctaggactgagctagctgtca

SEQ ID NO: 37 - DNA, 22 bp, synthetic construct
  source 1..22: mol_type = other DNA
caggcagttcattgagttagcg

SEQ ID NO: 38 - DNA, 45 bp, synthetic construct
  source 1..45: mol_type = other DNA
cacagtgtattaagcagacgttaaatacaaaaaatgggacggcac

SEQ ID NO: 39 - DNA, 73 bp, synthetic construct
  source 1..73: mol_type = other DNA
gttatccgctcacaattccacacattatacgagccggatgattaattgtcaattttatattccttttgcgctc

SEQ ID NO: 40 - DNA, 20 bp, synthetic construct
  source 1..20: mol_type = other DNA
acggttagggatggttcgac

SEQ ID NO: 41 - DNA, 45 bp, synthetic construct
  source 1..45: mol_type = other DNA
gtgccgtcccattttttgtatttaacgtctgcttaatacactgtg

SEQ ID NO: 42 - DNA, 76 bp, synthetic construct
  source 1..76: mol_type = other DNA
gtataatgtgtggaattgtgagcggataacaatttcacacaggaaacagaccatggaactttttaaatatatggag

SEQ ID NO: 43 - DNA, 91 bp, synthetic construct
  source 1..91: mol_type = other DNA
tgacagctagctcagtcctaggtataatactagtcgcccctcttatatcgcgctggggttttagagctagaaatagcaagttaaaataagg

SEQ ID NO: 44 - DNA, 91 bp, synthetic construct
  source 1..91: mol_type = other DNA
ccttattttaacttgctatttctagctctaaaaccccagcgcgatataagaggggcgactagtattatacctaggactgagctagctgtca

SEQ ID NO: 45 - DNA, 20 bp, synthetic construct
  source 1..20: mol_type = other DNA
ttctattcaggacgccaacg

SEQ ID NO: 46 - DNA, 43 bp, synthetic construct
  source 1..43: mol_type = other DNA
gctataacgcataaagtcacggcacgcttcctccttacgcagg

SEQ ID NO: 47 - DNA, 43 bp, synthetic construct
  source 1..43: mol_type = other DNA
cctgcgtaaggaggaagcgtgccgtgactttatgcgttatagc

SEQ ID NO: 48 - DNA, 22 bp, synthetic construct
  source 1..22: mol_type = other DNA
gcctgcaaagtgcccataaccc

SEQ ID NO: 49 - DNA, 91 bp, synthetic construct
  source 1..91: mol_type = other DNA
tgacagctagctcagtcctaggtataatactagtgcctttcagttccgcaacaaagggttttagagctagaaatagcaagttaaaataagg

SEQ ID NO: 50 - DNA, 91 bp, synthetic construct
  source 1..91: mol_type = other DNA
ccttattttaacttgctatttctagctctaaaaccctttgttgcggaactgaaaggcactagtattatacctaggactgagctagctgtca

SEQ ID NO: 51 - DNA, 20 bp, synthetic construct
  source 1..20: mol_type = other DNA
aacttcctccaaaccgatgc

SEQ ID NO: 52 - DNA, 45 bp, synthetic construct
  source 1..45: mol_type = other DNA
caatataataaggagtttaggttgattagcggataataaaaaacc

SEQ ID NO: 53 - DNA, 45 bp, synthetic construct
  source 1..45: mol_type = other DNA
ggttttttattatccgctaatcaacctaaactccttattatattg

SEQ ID NO: 54 - DNA, 20 bp, synthetic construct
  source 1..20: mol_type = other DNA
tcttcaatggactggaggtg